European Patent Specification EP 4 196 581 B1, published February 25, 2026. Title: SEQUENTIAL ENCODING METHODS AND RELATED KITS. Applicant: Encodia, Inc. The sequence listing filed with the application follows.

SEQUENCE LISTING (8 sequences)

SEQ ID NO: 1 - DNA, 20 bp, Artificial Sequence
  P5 primer
aatgatacggcgaccaccga

SEQ ID NO: 2 - DNA, 24 bp, Artificial Sequence
  P7 primer
caagcagaagacggcatacgagat

SEQ ID NO: 3 - protein, 19 aa, Artificial Sequence
  Test peptide
FAGVAMPGAEDDVVGSGSK

SEQ ID NO: 4 - protein, 20 aa, Artificial Sequence
  Test peptide
AFAGVAMPGAEDDVVGSGSK

SEQ ID NO: 5 - protein, 19 aa, Artificial Sequence
  Test peptide
AAGVAMPGAEDDVVGSGSK

SEQ ID NO: 6 - protein, 13 aa, Artificial Sequence
  F-peptide
  MISC_FEATURE (13)..(13): an azido substituent on the lysine side chain
FSGVARGDVRGGK

SEQ ID NO: 7 - protein, 18 aa, Artificial Sequence
  L-peptide
  MISC_FEATURE (18)..(18): an azido substituent on the lysine side chain
LAESAFSGVARGDVRGGK

SEQ ID NO: 8 - DNA, 53 bp, Artificial Sequence
  Capture DNA
  misc_feature (1)..(1): 5'-phosphorylated
  misc_feature (19)..(19): n is an internal 5'-amino modifier C6 dT
  misc_feature (20)..(21): C3 (three carbon) spacer inserted in between
tgtagggaaagagtgtttntacactctttccctacacgacgctcttccgatct